European Patent Application EP 4 428 239 A1, published September 11, 2024. Title: Novel anti-Nav1.7 monoclonal antibodies. Applicant: SHIONOGI & CO., LTD. The sequence listing filed with the application follows.

SEQUENCE LISTING (103 sequences)

SEQ ID NO: 1 - protein, 8 aa, synthetic construct
  REGION 1..8: note = hCE3C peptide
QPKYEYSL

SEQ ID NO: 2 - protein, 9 aa, synthetic construct
  REGION 1..9: note = N terminal Cys-added-hCE3C peptide
CQPKYEYSL

SEQ ID NO: 3 - protein, 119 aa, synthetic construct
  REGION 1..119: note = Heavy chain of 15H11
EVQLQQSGPELLKPGASVKISCKASGYTFTDYNMHWVKQSHGRSLEWIGRINPKNGVINSNEKFKDKATLTVDKSLSTAYMDLRSLTSEDSAVYFCAPSYYGGNTDAYWGHGTLVTVSA

SEQ ID NO: 4 - protein, 5 aa, synthetic construct
  REGION 1..5: note = CDR1 of 15H11 VH
DYNMH

SEQ ID NO: 5 - protein, 17 aa, synthetic construct
  REGION 1..17: note = CDR2 of 15H11 VH
RINPKNGVINSNEKFKD

SEQ ID NO: 6 - protein, 10 aa, synthetic construct
  REGION 1..10: note = CDR3 of 15H11 VH
SYYGGNTDAY

SEQ ID NO: 7 - protein, 113 aa, synthetic construct
  REGION 1..113: note = Light chain of 15H11
DIVLTQSPVSLAVSLGQRATIYCRASESVDNYGISFMNWFQQKPGQPPKLLIYAASSQGSGVPARFSGSGSGTDFSLNIHPMEEDDTAMYFCQQSKEFPWTFGGGTKLEIKRA

SEQ ID NO: 8 - protein, 15 aa, synthetic construct
  REGION 1..15: note = CDR1 of 15H11 VK
RASESVDNYGISFMN

SEQ ID NO: 9 - protein, 7 aa, synthetic construct
  REGION 1..7: note = CDR2 of 15H11 VK
AASSQGS

SEQ ID NO: 10 - protein, 9 aa, synthetic construct
  REGION 1..9: note = CDR3 of 15H11 VK
QQSKEFPWT

SEQ ID NO: 11 - protein, 327 aa, synthetic construct
  REGION 1..327: note = hIgG4Pro
ASTKGPSVFPLAPCSRSTSESTAALGCLVKDYFPEPVTVSWNSGALTSGVHTFPAVLQSSGLYSLSSVVTVPSSSLGTKTYTCNVDHKPSNTKVDKRVESKYGPPCPPCPAPEFLGGPSVFLFPPKPKDTLMISRTPEVTCVVVDVSQEDPEVQFNWYVDGVEVHNAKTKPREEQFNSTYRVVSVLTVLHQDWLNGKEYKCKVSNKGLPSSIEKTISKAKGQPREPQVYTLPPSQEEMTKNQVSLTCLVKGFYPSDIAVEWESNGQPENNYKTTPPVLDSDGSFFLYSRLTVDKSRWQEGNVFSCSVMHEALHNHYTQKSLSLSLGK

SEQ ID NO: 12 - protein, 105 aa, synthetic construct [sequence omitted]

SEQ ID NO: 13 - protein, 15 aa, synthetic construct
  REGION 1..15: note = Nav1.7 CE3C peptide
CSVNVDKQPKYEYSL

SEQ ID NO: 14 - protein, 113 aa, synthetic construct
  REGION 1..113: note = Light chain
DIVLTQSPASLAVSPGQRATITCRASESVDNYGISFMNWYQQKPGQPPKLLIYAASSQGSGVPARFSGSGSGTDFTLTINPVEANDTANYYCQQSKEFPWTFGGGTKVEIKRT

SEQ ID NO: 15 - protein, 113 aa, synthetic construct
  REGION 1..113: note = Light chain
DIQMTQSPSSLSASVGDRVTITCRASESVDNYGISFMNWYQQKPGKAPKLLIYAASSQGSGVPSRFSGSGSGTDFTLTISSLQPEDFATYYCQQSKEFPWTFGGGTKVEIKRT

SEQ ID NO: 16 - protein, 113 aa, synthetic construct
  REGION 1..113: note = Light chain
EIVLTQSPATLSLSPGERATLSCRASESVDNYGISFMNWYQQKPGQAPRLLIYAASSQGSGIPARFSGSGSGTDFTLTISSLEPEDFAVYYCQQSKEFPWTFGGGTKVEIKRT

SEQ ID NO: 17 - protein, 113 aa, synthetic construct
  REGION 1..113: note = Light chain
EIVLTQSPATLSLSPGERATLSCRASESVDNYGISFMNWYQQKPGQAPRLLIYAASSQGSGIPARFSGSGSGTDFTLTISRLEPEDFAVYYCQQSKEFPWTFGGGTKVEIKRT

SEQ ID NO: 18 - protein, 113 aa, synthetic construct
  REGION 1..113: note = Light chain
DIVMTQSPDSLAVSLGERATINCRASESVDNYGISFMNWYQQKPGQPPKLLIYAASSQGSGVPDRFSGSGSGTDFTLTISSLQAEDVAVYYCQQSKEFPWTFGGGTKVEIKRT

SEQ ID NO: 19 - protein, 119 aa, synthetic construct
  REGION 1..119: note = Heavy chain
QVQLVQSGAEVKKPGASVKVSCKASGYTFTDYNMHWVRQAPGQGLEWMGRINPKNGVINSNEKFKDRVTMTRDTSISTAYMELSRLRSDDTAVYYCARSYYGGNTDAYWGQGTLVTVSS

SEQ ID NO: 20 - protein, 119 aa, synthetic construct
  REGION 1..119: note = Heavy chain
QVQLVQSGAEVKKPGASVKVSCKASGYTFTDYNMHWVRQAPGQGLEWMGRINPKNGVINSNEKFKDRVTMTRDTSISTAYMELSRLRSDDTAVYYCAPSYYGGNTDAYWGQGTLVTVSS

SEQ ID NO: 21 - protein, 119 aa, synthetic construct
  REGION 1..119: note = Heavy chain
QVQLVQSGAEVKKPGASVKVSCKASGYTFTDYNMHWVRQAPGQRLEWMGRINPKNGVINSNEKFKDRVTITRDTSASTAYMELSSLRSEDTAVYYCAPSYYGGNTDAYWGQGTLVTVSS

SEQ ID NO: 22 - protein, 119 aa, synthetic construct
  REGION 1..119: note = Heavy chain
QVQLVQSGAEVKKPGASVKVSCKASGYTFTDYNMHWVRQAPGQGLEWMGRINPKNGVINSNEKFKDRVTMTTDTSTSTAYMELRSLRSDDTAVYYCAPSYYGGNTDAYWGQGTLVTVSS

SEQ ID NO: 23 - protein, 119 aa, synthetic construct
  REGION 1..119: note = Heavy chain
QVQLVQSGAEVKKPGASVKVSCKASGYTFTDYNMHWVRQAPGQGLEWMGRINPKNGVINSNEKFKDRVTMTRDTSTSTVYMELSSLRSEDTAVYYCAPSYYGGNTDAYWGQGTLVTVSS

SEQ ID NO: 24 - protein, 119 aa, synthetic construct
  REGION 1..119: note = Heavy chain
QVQLVQSGSELKKPGASVKVSCKASGYTFTDYNMHWVRQAPGQGLEWMGRINPKNGVINSNEKFKDRFVFSLDTSVSTAYLQISSLKAEDTAVYYCAPSYYGGNTDAYWGQGTLVTVSS

SEQ ID NO: 25 - protein, 119 aa, synthetic construct
  REGION 1..119: note = Heavy chain
QVQLVQSGSELKKPGASVKVSCKASGYTFTDYNMHWVRQAPGRSLEWMGRINPKNGVINSNEKFKDRFVFSLDTSVSTAYLQISSLKAEDTAVYYCAPSYYGGNTDAYWGQGTLVTVSS

SEQ ID NO: 26 - protein, 119 aa, synthetic construct
  REGION 1..119: note = Heavy chain
QVQLVQSGAEVKKPGASVKVSCKASGYTFTDYNMHWVRQAPGRSLEWMGRINPKNGVINSNEKFKDRVTMTRDTSISTAYMELSRLRSDDTAVYYCAPSYYGGNTDAYWGQGTLVTVSS

SEQ ID NO: 27 - protein, 113 aa, synthetic construct
  REGION 1..113: note = Light chain
DIVLTQSPASLAVSPGQRATITCRASESVDNYGISFMNWFQQKPGQPPKLLIYAASSQGSGVPARFSGSGSGTDFTLTINPMEANDTAMYYCQQSKEFPWTFGGGTKVEIKRT

SEQ ID NO: 28 - protein, 113 aa, synthetic construct
  REGION 1..113: note = Light chain
DIVLTQSPASLAVSPGQRATITCRASESVDNYGISFMNWFQQKPGQPPKLLIYAASSQGSGVPARFSGSGSGTDFTLTINPMEANDTANYYCQQSKEFPWTFGGGTKVEIKRT

SEQ ID NO: 29 - protein, 113 aa, synthetic construct
  REGION 1..113: note = Light chain
DIVLTQSPASLAVSPGQRATITCRASESVDNYGISFMNWFQQKPGQPPKLLIYAASSQGSGVPARFSGSGSGTDFTLTINPVEANDTAMYYCQQSKEFPWTFGGGTKVEIKRT

SEQ ID NO: 30 - protein, 113 aa, synthetic construct
  REGION 1..113: note = Light chain
DIVLTQSPASLAVSPGQRATITCRASESVDNYGISFMNWFQQKPGQPPKLLIYAASSQGSGVPARFSGSGSGTDFSLNINPVEANDTANYYCQQSKEFPWTFGGGTKVEIKRT

SEQ ID NO: 31 - protein, 113 aa, synthetic construct
  REGION 1..113: note = Light chain
DIVLTQSPASLAVSPGQRATITCRASESVDNYGISFMNWFQQKPGQPPKLLIYAASSQGSGVPARFSGSGSGTDFTLTINPVEANDTANYYCQQSKEFPWTFGGGTKVEIKRT

SEQ ID NO: 32 - protein, 119 aa, synthetic construct
  REGION 1..119: note = Heavy chain
QVQLVQSGSELKKPGASVKVSCKASGYTFTEYNMHWVRQAPGRSLEWMGRINPKNGVILSNEKFKDRFVFSLDTSVSTAYLQISSLKAEDTAVYYCAPSYYGGDDDAYWGQGTLVTVSS

SEQ ID NO: 33 - protein, 119 aa, synthetic construct
  REGION 1..119: note = Heavy chain
QVQLVQSGSELKKPGASVKVSCKASGYTFTDYNMHWVRQAPGRSLEWMGRINPKNGVILSNEKFKDRFVFSLDTSVSTAYLQISSLKAEDTAVYYCAPSYYGGDDDAYWGQGTLVTVSS

SEQ ID NO: 34 - protein, 119 aa, synthetic construct
  REGION 1..119: note = Heavy chain
QVQLVQSGSELKKPGASVKVSCKASGYTFTEYNMHWVRQAPGRSLEWMGRINPKNGVILSNEKFKDRFVFSLDTSVSTAYLQISSLKAEDTAVYYCAPSYYGGDTDAYWGQGTLVTVSS

SEQ ID NO: 35 - protein, 119 aa, synthetic construct
  REGION 1..119: note = Heavy chain
QVQLVQSGSELKKPGASVKVSCKASGYTFTDYNMHWVRQAPGRSLEWMGRINPKNGVINSNEKFKDRFVFSLDTSVSTAYLQISSLKAEDTAVYYCAPSYYGGDDDAYWGQGTLVTVSS

SEQ ID NO: 36 - protein, 119 aa, synthetic construct
  REGION 1..119: note = Heavy chain
QVQLVQSGSELKKPGASVKVSCKASGYTFTEYNMHWVRQAPGRSLEWMGRINPKNGVILSNEKFKDRFVFSLDTSVSTAYLQISSLKAEDTAVYYCAPSYYGGNDDAYWGQGTLVTVSS

SEQ ID NO: 37 - protein, 119 aa, synthetic construct
  REGION 1..119: note = Heavy chain
QVQLVQSGSELKKPGASVKVSCKASGYTFTDYNMHWVRQAPGRSLEWMGRINPKNGVILSNEKFKDRFVFSLDTSVSTAYLQISSLKAEDTAVYYCAPSYYGGNDDAYWGQGTLVTVSS

SEQ ID NO: 38 - protein, 119 aa, synthetic construct
  REGION 1..119: note = Heavy chain
QVQLVQSGSELKKPGASVKVSCKASGYTFTDYNMHWVRQAPGRSLEWMGRINPKNGVILSNEKFKDRFVFSLDTSVSTAYLQISSLKAEDTAVYYCAPSYYGGDTDAYWGQGTLVTVSS

SEQ ID NO: 39 - protein, 119 aa, synthetic construct
  REGION 1..119: note = Heavy chain
QVQLVQSGSELKKPGASVKVSCKASGYTFTEYNMHWVRQAPGRSLEWMGRINPKNGVINSNEKFKDRFVFSLDTSVSTAYLQISSLKAEDTAVYYCAPSYYGGNDDAYWGQGTLVTVSS

SEQ ID NO: 40 - protein, 119 aa, synthetic construct
  REGION 1..119: note = Heavy chain
QVQLVQSGSELKKPGASVKVSCKASGYTFTDYNMHWVRQAPGRSLEWMGRINPKNGVINSNEKFKDRFVFSLDTSVSTAYLQISSLKAEDTAVYYCAPSYYGGNDDAYWGQGTLVTVSS

SEQ ID NO: 41 - protein, 119 aa, synthetic construct
  REGION 1..119: note = Heavy chain
QVQLVQSGSELKKPGASVKVSCKASGYTFTEYNMHWVRQAPGRSLEWMGRINPKNGVINSNEKFKDRFVFSLDTSVSTAYLQISSLKAEDTAVYYCAPSYYGGDTDAYWGQGTLVTVSS

SEQ ID NO: 42 - protein, 119 aa, synthetic construct
  REGION 1..119: note = Heavy chain
QVQLVQSGSELKKPGASVKVSCKASGYTFTEYNMHWVRQAPGRSLEWMGRINPKNGVILSNEKFKDRFVFSLDTSVSTAYLQISSLKAEDTAVYYCAPSYYGGNTDAYWGQGTLVTVSS

SEQ ID NO: 43 - protein, 119 aa, synthetic construct
  REGION 1..119: note = Heavy chain
QVQLVQSGSELKKPGASVKVSCKASGYTFTEYNMHWVRQAPGRSLEWMGRINPKNGVINSNEKFKDRFVFSLDTSVSTAYLQISSLKAEDTAVYYCAPSYYGGNSDAYWGQGTLVTVSS

SEQ ID NO: 44 - protein, 119 aa, synthetic construct
  REGION 1..119: note = Heavy chain
QVQLVQSGSELKKPGASVKVSCKASGYTFTEYNMHWVRQAPGRSLEWMGRINPKNGVIQSNEKFKDRFVFSLDTSVSTAYLQISSLKAEDTAVYYCAPSYYGGNSDAYWGQGTLVTVSS

SEQ ID NO: 45 - protein, 119 aa, synthetic construct
  REGION 1..119: note = Heavy chain
QVQLVQSGSELKKPGASVKVSCKASGYTFTDYNMHWVRQAPGRSLEWMGRINPKNGVINSNEKFKDRFVFSLDTSVSTAYLQISSLKAEDTAVYYCAPSYYGGDTDAYWGQGTLVTVSS

SEQ ID NO: 46 - protein, 119 aa, synthetic construct
  REGION 1..119: note = Heavy chain
QVQLVQSGSELKKPGASVKVSCKASGYTFTDYNMHWVRQAPGRSLEWMGRINPKNGVILSNEKFKDRFVFSLDTSVSTAYLQISSLKAEDTAVYYCAPSYYGGNTDAYWGQGTLVTVSS

SEQ ID NO: 47 - protein, 119 aa, synthetic construct
  REGION 1..119: note = Heavy chain
QVQLVQSGSELKKPGASVKVSCKASGYTFTDYNMHWVRQAPGRSLEWMGRINPKNGVIQSNEKFKDRFVFSLDTSVSTAYLQISSLKAEDTAVYYCAPSYYGGNSDAYWGQGTLVTVSS

SEQ ID NO: 48 - protein, 119 aa, synthetic construct
  REGION 1..119: note = Heavy chain
QVQLVQSGSELKKPGASVKVSCKASGYTFTEYNMHWVRQAPGRSLEWMGRINPKNGVINSNEKFKDRFVFSLDTSVSTAYLQISSLKAEDTAVYYCAPSYFGGQSDAYWGQGTLVTVSS

SEQ ID NO: 49 - protein, 119 aa, synthetic construct
  REGION 1..119: note = Heavy chain
QVQLVQSGSELKKPGASVKVSCKASGYTFTDYNMHWVRQAPGRSLEWMGRINPKNGVINSNEKFKDRFVFSLDTSVSTAYLQISSLKAEDTAVYYCAPSYYGGNQDAYWGQGTLVTVSS

SEQ ID NO: 50 - protein, 119 aa, synthetic construct
  REGION 1..119: note = Heavy chain
QVQLVQSGSELKKPGASVKVSCKASGYTFTDYNMHWVRQAPGRSLEWMGRINPKNGVINLNEKFKDRFVFSLDTSVSTAYLQISSLKAEDTAVYYCAPSYYGGNTDAYWGQGTLVTVSS

SEQ ID NO: 51 - protein, 119 aa, synthetic construct
  REGION 1..119: note = Heavy chain
QVQLVQSGSELKKPGASVKVSCKASGYTFTDYNMHWVRQAPGRSLEWMGRINPKNGVIKSNEKFKDRFVFSLDTSVSTAYLQISSLKAEDTAVYYCAPSYYGGNTDAYWGQGTLVTVSS

SEQ ID NO: 52 - protein, 119 aa, synthetic construct
  REGION 1..119: note = Heavy chain
QVQLVQSGSELKKPGASVKVSCKASGYTFTDYNMHWVRQAPGRSLEWMGRINPKNGVINYNEKFKDRFVFSLDTSVSTAYLQISSLKAEDTAVYYCAPSYYGGNTDAYWGQGTLVTVSS

SEQ ID NO: 53 - protein, 119 aa, synthetic construct
  REGION 1..119: note = Heavy chain
QVQLVQSGSELKKPGASVKVSCKASGYTFTDYNMHWVRQAPGRSLEWMGRINPKNGVINSNEKFKDRFVFSLDTSVSTAYLQISSLKAEDTAVYYCAPSYFGGNSDAYWGQGTLVTVSS

SEQ ID NO: 54 - protein, 119 aa, synthetic construct
  REGION 1..119: note = Heavy chain
QVQLVQSGSELKKPGASVKVSCKASGYTFTDYNMHWVRQAPGRSLEWMGRINPKNGVINSNEKFKDRFVFSLDTSVSTAYLQISSLKAEDTAVYYCAPSYYGGKTDAYWGQGTLVTVSS

SEQ ID NO: 55 - protein, 113 aa, synthetic construct
  REGION 1..113: note = Light chain
DIVLTQSPASLAVSPGQRATITCRASDSVDNYGISFLNWFQQKPGQPPKLLIYAASSQGSGVPARFSGSGSGTDFTLTINPMEANDTANYYCQQSKEFPWTFGGGTKVEIKRT

SEQ ID NO: 56 - protein, 113 aa, synthetic construct
  REGION 1..113: note = Light chain
DIVLTQSPASLAVSPGQRATITCRVSDSVDNYGISFLNWFQQKPGQPPKLLIYAASSQGSGVPARFSGSGSGTDFTLTINPMEANDTANYYCQQSKEFPWTFGGGTKVEIKRT

SEQ ID NO: 57 - protein, 113 aa, synthetic construct
  REGION 1..113: note = Light chain
DIVLTQSPASLAVSPGQRATITCRASESVDNYGFSFMNWFQQKPGQPPKLLIYAASSQGSGVPARFSGSGSGTDFTLTINPMEANDTANYYCQQSKEFPWTFGGGTKVEIKRT

SEQ ID NO: 58 - protein, 5 aa, synthetic construct
  REGION 1..5: note = mutant CDR1 of 15H11 VH
EYNMH

SEQ ID NO: 59 - protein, 17 aa, synthetic construct
  REGION 1..17: note = mutant CDR2 of 15H11 VH
RINPKNGVILSNEKFKD

SEQ ID NO: 60 - protein, 17 aa, synthetic construct
  REGION 1..17: note = mutant CDR2 of 15H11 VH
RINPKNGVIQSNEKFKD

SEQ ID NO: 61 - protein, 17 aa, synthetic construct
  REGION 1..17: note = mutant CDR2 of 15H11 VH
RINPKNGVINLNEKFKD

SEQ ID NO: 62 - protein, 17 aa, synthetic construct
  REGION 1..17: note = mutant CDR2 of 15H11 VH
RINPKNGVIKSNEKFKD

SEQ ID NO: 63 - protein, 17 aa, synthetic construct
  REGION 1..17: note = mutant CDR2 of 15H11 V
RINPKNGVINYNEKFKD

SEQ ID NO: 64 - protein, 10 aa, synthetic construct
  REGION 1..10: note = mutant CDR3 of 15H11 VH
SYYGGDDDAY

SEQ ID NO: 65 - protein, 10 aa, synthetic construct
  REGION 1..10: note = mutant CDR3 of 15H11 VH
SYYGGDTDAY

SEQ ID NO: 66 - protein, 10 aa, synthetic construct
  REGION 1..10: note = mutant CDR3 of 15H11 VH
SYYGGNDDAY

SEQ ID NO: 67 - protein, 10 aa, synthetic construct
  REGION 1..10: note = mutant CDR3 of 15H11 VH
SYYGGNSDAY

SEQ ID NO: 68 - protein, 10 aa, synthetic construct
  REGION 1..10: note = mutant CDR3 of 15H11 VH
SYFGGQSDAY

SEQ ID NO: 69 - protein, 10 aa, synthetic construct
  REGION 1..10: note = mutant CDR3 of 15H11 VH
SYYGGNQDAY

SEQ ID NO: 70 - protein, 10 aa, synthetic construct
  REGION 1..10: note = mutant CDR3 of 15H11 VH
SYFGGNSDAY

SEQ ID NO: 71 - protein, 10 aa, synthetic construct
  REGION 1..10: note = mutant CDR3 of 15H11 VH
SYYGGKTDAY

SEQ ID NO: 72 - protein, 15 aa, synthetic construct
  REGION 1..15: note = mutant CDR1 of 15H11 VK
RASDSVDNYGISFLN

SEQ ID NO: 73 - protein, 15 aa, synthetic construct
  REGION 1..15: note = mutant CDR1 of 15H11 VK
RVSDSVDNYGISFLN

SEQ ID NO: 74 - protein, 15 aa, synthetic construct
  REGION 1..15: note = mutant CDR1 of 15H11 VK
RASESVDNYGFSFMN

SEQ ID NO: 75 - protein, 5 aa, synthetic construct
  REGION 1..5: note = CDR1 of 15H11 VH
  SITE 1: note = X can be D or E.
XYNMH

SEQ ID NO: 76 - protein, 17 aa, synthetic construct
  REGION 1..17: note = CDR2 of 15H11 VH
  SITE 10: note = X can be N, L, Q or K.
  SITE 11: note = X can be S, L or Y.
RINPKNGVIXXNEKFKD

SEQ ID NO: 77 - protein, 10 aa, synthetic construct
  REGION 1..10: note = CDR3 of 15H11 VH
  SITE 3: note = X can be Y or F.
  SITE 6: note = X can be N, D, Q or K.
  SITE 7: note = X can be T, D, S or Q.
SYXGGXXDAY

SEQ ID NO: 78 - protein, 15 aa, synthetic construct
  REGION 1..15: note = CDR1 of 15H11 VK
  SITE 2: note = X can be A or V.
  SITE 4: note = X can be E or D.
  SITE 11: note = X can be I or F.
  SITE 14: note = X can be M or L.
RXSXSVDNYGXSFXN

SEQ ID NO: 79 - protein, 113 aa, synthetic construct
  REGION 1..113: note = Light chain
DIVLTQSPASLAVSPGQRATITCRASDSVDNYGISFLNWFQQKPGQPPKLLIYAASSQGSGVPARFSGSGSGTDFTLTINPMEAEDTANYYCQQSKEFPWTFGGGTKVEIKRT

SEQ ID NO: 80 - protein, 113 aa, synthetic construct
  REGION 1..113: note = Light chain
DIVLTQSPASLAVSPGQRATITCRASDSVDNYGISFLNWFQQKPGQPPKLLIYAASSQGSGVPARFSGSGSGTDFTLTINPMEAADTANYYCQQSKEFPWTFGGGTKVEIKRT

SEQ ID NO: 81 - protein, 113 aa, synthetic construct
  REGION 1..113: note = Light chain
DIVLTQSPASLAVSPGQRATITCRASDSVDNYGISFLNWFQQKPGQPPKLLIYAASSQGSGVPARFSGSGSGTDFTLTINPMEAQDTANYYCQQSKEFPWTFGGGTKVEIKRT

SEQ ID NO: 82 - protein, 113 aa, synthetic construct
  REGION 1..113: note = Light chain
DIVLTQSPASLAVSPGQRATITCRASDSVDNYGISFLNWFQQKPGQPPKLLIYAASSQGSGVPARFSGSGSGTDFTLTINPMEAFDTANYYCQQSKEFPWTFGGGTKVEIKRT

SEQ ID NO: 83 - protein, 113 aa, synthetic construct
  REGION 1..113: note = Light chain
DIVLTQSPASLAVSPGQRATITCRASDSVDNYGISFLNWFQQKPGQPPKLLIYAASSQGSGVPARFSGSGSGTDFTLTINPMEALDTANYYCQQSKEFPWTFGGGTKVEIKRT

SEQ ID NO: 84 - protein, 113 aa, synthetic construct
  REGION 1..113: note = Light chain
DIVLTQSPASLAVSPGQRATITCRASDSVDNYGISFLNWFQQKPGQPPKLLIYAASSQGSGVPARFSGSGSGTDFTLTINPMEAVDTANYYCQQSKEFPWTFGGGTKVEIKRT

SEQ ID NO: 85 - protein, 113 aa, synthetic construct
  REGION 1..113: note = Light chain
DIVLTQSPASLAVSPGQRATITCRASDSVDNYGISFLNWFQQKPGQPPKLLIYAASSQGSGVPARFSGSGSGTDFTLTINPMEAIDTANYYCQQSKEFPWTFGGGTKVEIKRT

SEQ ID NO: 86 - protein, 113 aa, synthetic construct
  REGION 1..113: note = Light chain
DIVLTQSPASLAVSPGQRATITCRASDSVDNYGISFLNWFQQKPGQPPKLLIYAASSQGSGVPARFSGSGSGTDFTLTINPMEADDTANYYCQQSKEFPWTFGGGTKVEIKRT

SEQ ID NO: 87 - protein, 113 aa, synthetic construct
  REGION 1..113: note = Light chain
DIVLTQSPASLAVSPGQRATITCRASDSVDNYGISFLNWFQQKPGQPPKLLIYAASSQGSGVPARFSGSGSGTDFTLTINPMEARDTANYYCQQSKEFPWTFGGGTKVEIKRT

SEQ ID NO: 88 - protein, 113 aa, synthetic construct
  REGION 1..113: note = Light chain
DIVLTQSPASLAVSPGQRATITCRASDSVDNYGISFLNWFQQKPGQPPKLLIYAASSQGSGVPARFSGSGSGTDFTLTINPMEAGDTANYYCQQSKEFPWTFGGGTKVEIKRT

SEQ ID NO: 89 - protein, 113 aa, synthetic construct
  REGION 1..113: note = Light chain
DIVLTQSPASLAVSPGQRATITCRASDSVDNYGISFLNWFQQKPGQPPKLLIYAASSQGSGVPARFSGSGSGTDFTLTINPMEANPTANYYCQQSKEFPWTFGGGTKVEIKRT

SEQ ID NO: 90 - protein, 113 aa, synthetic construct
  REGION 1..113: note = Light chain
DIVMTQSPDSLAVSLGERATINCRASESVDNYGISFMNWFQQKPGQPPKLLIYAASSQGSGVPDRFSGSGSGTDFTLTISSMQAEDVAMYYCQQSKEFPWTFGGGTKVEIKRT

SEQ ID NO: 91 - protein, 113 aa, synthetic construct
  REGION 1..113: note = Light chain
DIVMTQSPDSLAVSLGERATINCRASESVDNYGISFMNWFQQKPGQPPKLLIYAASSQGSGVPDRFSGSGSGTDFTLTINPMQAEDVAVYYCQQSKEFPWTFGGGTKVEIKRT

SEQ ID NO: 92 - protein, 113 aa, synthetic construct
  REGION 1..113: note = Light chain
DIVMTQSPDSLAVSLGERATINCRASESVDNYGISFMNWFQQKPGQPPKLLIYAASSQGSGVPDRFSGSGSGTDFTLTISSMQAEDVAVYYCQQSKEFPWTFGGGTKVEIKRT

SEQ ID NO: 93 - protein, 113 aa, synthetic construct
  REGION 1..113: note = Light chain
DIVMTQSPDSLAVSLGERATINCRASDSVDNYGISFLNWFQQKPGQPPKLLIYAASSQGSGVPDRFSGSGSGTDFTLTISSMQAEDVAMYYCQQSKEFPWTFGGGTKVEIKRT

SEQ ID NO: 94 - protein, 113 aa, synthetic construct
  REGION 1..113: note = Light chain
DIVMTQSPDSLAVSLGERATINCRASDSVDNYGISFLNWFQQKPGQPPKLLIYAASSQGSGVPDRFSGSGSGTDFTLTINPMQAEDVAVYYCQQSKEFPWTFGGGTKVEIKRT

SEQ ID NO: 95 - protein, 113 aa, synthetic construct
  REGION 1..113: note = Light chain
DIVMTQSPDSLAVSLGERATINCRASDSVDNYGISFLNWFQQKPGQPPKLLIYAASSQGSGVPDRFSGSGSGTDFTLTISSMQAEDVAVYYCQQSKEFPWTFGGGTKVEIKRT

SEQ ID NO: 96 - protein, 113 aa, synthetic construct
  REGION 1..113: note = Light chain
DIVMTQSPDSLAVSLGERATINCRASDSVDNYGISFLNWFQQKPGQPPKLLIYAASSQGSGVPDRFSGSGSGTDFTLTINPMEAEDTANYYCQQSKEFPWTFGGGTKVEIKRT

SEQ ID NO: 97 - protein, 113 aa, synthetic construct
  REGION 1..113: note = Light chain
DIVMTQSPDSLAVSLGERATINCRASDSVDNYGISFLNWFQQKPGQPPKLLIYAASSQGSGVPDRFSGSGSGTDFTLTISSMEAEDVAVYYCQQSKEFPWTFGGGTKVEIKRT

SEQ ID NO: 98 - protein, 113 aa, synthetic construct
  REGION 1..113: note = Light chain
DIVMTQSPDSLAVSLGERATINCRASDSVDNYGISFLNWFQQKPGQPPKLLIYAASSQGSGVPDRFSGSGSGTDFTLTISSMQAEDTAVYYCQQSKEFPWTFGGGTKVEIKRT

SEQ ID NO: 99 - protein, 113 aa, synthetic construct
  REGION 1..113: note = Light chain
DIVMTQSPDSLAVSLGERATINCRASDSVDNYGISFLNWFQQKPGQPPKLLIYAASSQGSGVPARFSGSGSGTDFTLTISSMQAEDVAVYYCQQSKEFPWTFGGGTKVEIKRT

SEQ ID NO: 100 - protein, 113 aa, synthetic construct
  REGION 1..113: note = Light chain
DIVMTQSPDSLAVSLGERATINCRASDSVDNYGISFLNWFQQKPGQPPKLLIYAASSQGSGVPARFSGSGSGTDFTLTISSMQAEDVAMYYCQQSKEFPWTFGGGTKVEIKRT

SEQ ID NO: 101 - protein, 113 aa, synthetic construct
  REGION 1..113: note = Light chain
DIVLTQSPASLAVSLGERATINCRASDSVDNYGISFLNWFQQKPGQPPKLLIYAASSQGSGVPARFSGSGSGTDFTLTISSMQAEDVAVYYCQQSKEFPWTFGGGTKVEIKRT

SEQ ID NO: 102 - protein, 113 aa, synthetic construct
  REGION 1..113: note = Light chain
DIVLTQSPASLAVSLGQRATINCRASDSVDNYGISFLNWFQQKPGQPPKLLIYAASSQGSGVPARFSGSGSGTDFTLTISSMQAEDVAVYYCQQSKEFPWTFGGGTKVEIKRT

SEQ ID NO: 103 - protein, 14 aa, synthetic construct
  REGION 1..14: note = hCE3C peptide
SVNVDKQPKYEYSL